European Patent Application EP 4 467 560 A1, published November 27, 2024. Title: Peptide for atopic dermatitis prevention or treatment. Applicant: REMEDI CO., LTD. Application KR. The sequence listing filed with the application follows.

SEQUENCE LISTING (40 sequences)

SEQ ID NO: 1 - protein, 15 aa, Homo sapiens
LEKHSGKRRKKRRHR

SEQ ID NO: 2 - protein, 10 aa, Homo sapiens
GKRRKKRRHR

SEQ ID NO: 3 - protein, 12 aa, Homo sapiens
HSGKRRKKRRHR

SEQ ID NO: 4 - protein, 12 aa, Homo sapiens
GKRRKKRRHRSK

SEQ ID NO: 5 - protein, 12 aa, Homo sapiens
LEKHSGKRRKKR

SEQ ID NO: 6 - protein, 19 aa, Homo sapiens
LEKHSGKRRKKRRHRSKVN

SEQ ID NO: 7 - protein, 18 aa, Homo sapiens
NSTLEKHSGKRRKKRRHR

SEQ ID NO: 8 - protein, 22 aa, Homo sapiens
DVENNSTLEKHSGKRRKKRRHR

SEQ ID NO: 9 - protein, 19 aa, Homo sapiens
GKRRKKRRHRSKVNGLQRG

SEQ ID NO: 10 - protein, 12 aa, Homo sapiens
DVENNSTLEKHS

SEQ ID NO: 11 - protein, 19 aa, Homo sapiens
DVENNSTLEKHSGKRRKKR

SEQ ID NO: 12 - protein, 5 aa, Homo sapiens
LEKHS

SEQ ID NO: 13 - protein, 9 aa, Homo sapiens
LEKHSGKRR

SEQ ID NO: 14 - DNA, 20 bp, synthetic construct
  source 1..20: mol_type = other DNA
aagtggcatagatgtggaag

SEQ ID NO: 15 - DNA, 20 bp, synthetic construct
  source 1..20: mol_type = other DNA
gaatgcatcctttttcgcct

SEQ ID NO: 16 - DNA, 21 bp, synthetic construct
  source 1..21: mol_type = other DNA
cttgagcctagtcgtgataac

SEQ ID NO: 17 - DNA, 20 bp, synthetic construct
  source 1..20: mol_type = other DNA
ccagcttggtgaggtctatc

SEQ ID NO: 18 - DNA, 18 bp, synthetic construct
  source 1..18: mol_type = other DNA
cagagccaacgtcaagca

SEQ ID NO: 19 - DNA, 18 bp, synthetic construct
  source 1..18: mol_type = other DNA
aggtactcttggatccac

SEQ ID NO: 20 - DNA, 22 bp, synthetic construct
  source 1..22: mol_type = other DNA
ttgaagaagagcccatcctctg

SEQ ID NO: 21 - DNA, 20 bp, synthetic construct
  source 1..20: mol_type = other DNA
gatccacactctccagctgc

SEQ ID NO: 22 - DNA, 20 bp, synthetic construct
  source 1..20: mol_type = other DNA
accacggccttccctacttc

SEQ ID NO: 23 - DNA, 21 bp, synthetic construct
  source 1..21: mol_type = other DNA
ctcatttccacgatttcccag

SEQ ID NO: 24 - DNA, 22 bp, synthetic construct
  source 1..22: mol_type = other DNA
tgcccacgtcaaggagtatttc

SEQ ID NO: 25 - DNA, 22 bp, synthetic construct
  source 1..22: mol_type = other DNA
aacccacttcttctctgggttg

SEQ ID NO: 26 - DNA, 20 bp, synthetic construct
  source 1..20: mol_type = other DNA
atacagctgccgtgtttcag

SEQ ID NO: 27 - DNA, 21 bp, synthetic construct
  source 1..21: mol_type = other DNA
agccatcttatcacccaagaa

SEQ ID NO: 28 - DNA, 23 bp, synthetic construct
  source 1..23: mol_type = other DNA
accaactgggacgacatggagaa

SEQ ID NO: 29 - DNA, 20 bp, synthetic construct
  source 1..20: mol_type = other DNA
gtggtggtgaagctgtagcc

SEQ ID NO: 30 - DNA, 20 bp, synthetic construct
  source 1..20: mol_type = other DNA
ctgaaagcatgatccgggac

SEQ ID NO: 31 - DNA, 20 bp, synthetic construct
  source 1..20: mol_type = other DNA
ttagagagaggtccctgggg

SEQ ID NO: 32 - DNA, 20 bp, synthetic construct
  source 1..20: mol_type = other DNA
ctctgtgtgaaggtgcagtt

SEQ ID NO: 33 - DNA, 21 bp, synthetic construct
  source 1..21: mol_type = other DNA
ggggtggaaaggtttggagta

SEQ ID NO: 34 - DNA, 20 bp, synthetic construct
  source 1..20: mol_type = other DNA
cagtcgtctttgtcacccga

SEQ ID NO: 35 - DNA, 20 bp, synthetic construct
  source 1..20: mol_type = other DNA
cgggtggggtaggatagtga

SEQ ID NO: 36 - DNA, 19 bp, synthetic construct
  source 1..19: mol_type = other DNA
atggccccactgaagatgc

SEQ ID NO: 37 - DNA, 20 bp, synthetic construct
  source 1..20: mol_type = other DNA
aaaacgatggcatccctgga

SEQ ID NO: 38 - DNA, 20 bp, synthetic construct
  source 1..20: mol_type = other DNA
atcgcctacagactgcactc

SEQ ID NO: 39 - DNA, 21 bp, synthetic construct
  source 1..21: mol_type = other DNA
tcggcacagatctccttatcc

SEQ ID NO: 40 - protein, 31 aa, Homo sapiens
DVENNSTLEKHSGKRRKKRRHRSKVNGLQRG